European Patent Application EP 4 501 359 A1, published February 5, 2025. Title: Lipid nanoparticle. Applicant: NATIONAL UNIVERSITY CORPORATION HOKKAIDO UNIVERSITY. The sequence listing filed with the application follows.

SEQUENCE LISTING (26 sequences)

SEQ ID NO: 1 - RNA, 100 nt, synthetic construct
  source 1..100: mol_type = other RNA
ttacagccacgtctacagcagttttagagctagaaatagcaagttaaaataaggctagtccgttatcaacttgaaaaagtggcaccgagtcggtgctttt

SEQ ID NO: 2 - RNA, 100 nt, synthetic construct
  source 1..100: mol_type = other RNA
cccatactcctacagcaccagttttagagctagaaatagcaagttaaaataaggctagtccgttatcaacttgaaaaagtggcaccgagtcggtgctttt

SEQ ID NO: 3 - DNA, 132 bp, synthetic construct
  source 1..132: mol_type = other DNA
aaaaaaaaaaaaaaaaaaaaaaaaaaaaaaaaaaaaaaaaaaaaaaaaaaaaaaaatgctgtagacgtggctgtaaaaaaaaaaaaaaaaaaaaaaaaaaaaaaaaaaaaaaaaaaaaaaaaaaaaaaaaaa

SEQ ID NO: 4 - DNA, 132 bp, synthetic construct
  source 1..132: mol_type = other DNA
aaaaaaaaaaaaaaaaaaaaaaaaaaaaaaaaaaaaaaaaaaaaaaaaaaaaaaaaaactgtagacgtggctgtttaaaaaaaaaaaaaaaaaaaaaaaaaaaaaaaaaaaaaaaaaaaaaaaaaaaaaaaa

SEQ ID NO: 5 - DNA, 132 bp, synthetic construct
  source 1..132: mol_type = other DNA
aaaaaaaaaaaaaaaaaaaaaaaaaaaaaaaaaaaaaaaaaaaaaaaaaaaaaaaaaaaagtagacgtggctaattaaaaaaaaaaaaaaaaaaaaaaaaaaaaaaaaaaaaaaaaaaaaaaaaaaaaaaaa

SEQ ID NO: 6 - DNA, 132 bp, synthetic construct
  source 1..132: mol_type = other DNA
aaaaaaaaaaaaaaaaaaaaaaaaaaaaaaaaaaaaaaaaaaaaaaaaaaaaaaaaaaaaatagacgtggcaaattaaaaaaaaaaaaaaaaaaaaaaaaaaaaaaaaaaaaaaaaaaaaaaaaaaaaaaaa

SEQ ID NO: 7 - DNA, 132 bp, synthetic construct
  source 1..132: mol_type = other DNA
aaaaaaaaaaaaaaaaaaaaaaaaaaaaaaaaaaaaaaaaaaaaaaaaaaaaaaaaaaaaaaagacgtggaaaattaaaaaaaaaaaaaaaaaaaaaaaaaaaaaaaaaaaaaaaaaaaaaaaaaaaaaaaa

SEQ ID NO: 8 - DNA, 132 bp, synthetic construct
  source 1..132: mol_type = other DNA
aaaaaaaaaaaaaaaaaaaaaaaaaaaaaaaaaaaaaaaaaaaaaaaaaaaaaaaaaaaaaatgacgtgaaaaattaaaaaaaaaaaaaaaaaaaaaaaaaaaaaaaaaaaaaaaaaaaaaaaaaaaaaaaa

SEQ ID NO: 9 - DNA, 132 bp, synthetic construct
  source 1..132: mol_type = other DNA
aaaaaaaaaaaaaaaaaaaaaaaaaaaaaaaaaaaaaaaaaaaaaaaaaaaaaaaaaaaaaatataaaaaaaaattaaaaaaaaaaaaaaaaaaaaaaaaaaaaaaaaaaaaaaaaaaaaaaaaaaaaaaaa

SEQ ID NO: 10 - DNA, 132 bp, synthetic construct
  source 1..132: mol_type = other DNA
aaaaaaaaaaaaaaaaaaaaaaaaaaaaaaaaaaaaaaaaaaaaaaaaaaaaaaaaaagtgctgtaggagtatgaaaaaaaaaaaaaaaaaaaaaaaaaaaaaaaaaaaaaaaaaaaaaaaaaaaaaaaaaa

SEQ ID NO: 11 - DNA, 132 bp, synthetic construct
  source 1..132: mol_type = other DNA
aaaaaaaaaaaaaaaaaaaaaaaaaaaaaaaaaaaaaaaaaaaaaaaaaaaaaaaaaaaagctgtaggagtaaaaaaaaaaaaaaaaaaaaaaaaaaaaaaaaaaaaaaaaaaaaaaaaaaaaaaaaaaaaa

SEQ ID NO: 12 - DNA, 132 bp, synthetic construct; identical to SEQ ID NO: 3
  source 1..132: mol_type = other DNA

SEQ ID NO: 13 - DNA, 132 bp, synthetic construct
  source 1..132: mol_type = other DNA
aaaaaaaaaaaaaaaaaaaaaaaaaaaaaaaaaaaaaaaaaaaaaaaaaaaaaaaaaaaaaatgtaggagataaaaaaaaaaaaaaaaaaaaaaaaaaaaaaaaaaaaaaaaaaaaaaaaaaaaaaaaaaaa

SEQ ID NO: 14 - DNA, 132 bp, synthetic construct
  source 1..132: mol_type = other DNA
aaaaaaaaaaaaaaaaaaaaaaaaaaaaaaaaaaaaaaaaaaaaaaaaaaaaaaaaaaaaaaagtaggaaataaaaaaaaaaaaaaaaaaaaaaaaaaaaaaaaaaaaaaaaaaaaaaaaaaaaaaaaaaaa

SEQ ID NO: 15 - DNA, 132 bp, synthetic construct
  source 1..132: mol_type = other DNA
aaaaaaaaaaaaaaaaaaaaaaaaaaaaaaaaaaaaaaaaaaaaaaaaaaaaaaaaaaaaaaaaaaaaaaaaaaaaaaaaaaaaaaaaaaaaaaaaaaaaaaaaaaaaaaaaaaaaaaaaaaaaaaaaaaaa

SEQ ID NO: 16 - DNA, 132 bp, synthetic construct
  source 1..132: mol_type = other DNA
aaaaaaaaaaaaaaaaaaaaaaaaaaaaaaaaaaaaaaaaaaaaaaaaaaaaaaaaaaaaaatataaaaaaagtaaaaaaaaaaaaaaaaaaaaaaaaaaaaaaaaaaaaaaaaaaaaaaaaaaaaaaaaaa

SEQ ID NO: 17 - DNA, 132 bp, synthetic construct
  source 1..132: mol_type = other DNA
aaaaaaaaaaaaaaaaaaaaaaaaaaaaaaaaaaaaaaaaaaaaaaaaaaaaaaaatgcaaatataaaaaaaaattaaaaaaaaaaaaaaaaaaaaaaaaaaaaaaaaaaaaaaaaaaaaaaaaaaaaaaaa

SEQ ID NO: 18 - DNA, 132 bp, synthetic construct
  source 1..132: mol_type = other DNA
aaaaaaaaaaaaaaaaaaaaaaaaaaaaaaaaaaaaaaaaaaaaaaaaaaaaaaaaaaaaaatataaaggctgtaaaaaaaaaaaaaaaaaaaaaaaaaaaaaaaaaaaaaaaaaaaaaaaaaaaaaaaaaa

SEQ ID NO: 19 - DNA, 132 bp, synthetic construct
  source 1..132: mol_type = other DNA
aaaaaaaaaaaaaaaaaaaaaaaaaaaaaaaaaaaaaaaaaaaaaaaaaaaaaaaatgctgtagtaaaaaaaaattaaaaaaaaaaaaaaaaaaaaaaaaaaaaaaaaaaaaaaaaaaaaaaaaaaaaaaaa

SEQ ID NO: 20 - DNA, 132 bp, synthetic construct
  source 1..132: mol_type = other DNA
aaaaaaaaaaaaaaaaaaaaaaaaaaaaaaaaaaaaaaaaaaaaaaaaaaaaaaaatgctgtagacgtggctaattaaaaaaaaaaaaaaaaaaaaaaaaaaaaaaaaaaaaaaaaaaaaaaaaaaaaaaaa

SEQ ID NO: 21 - DNA, 132 bp, synthetic construct
  source 1..132: mol_type = other DNA
aaaaaaaaaaaaaaaaaaaaaaaaaaaaaaaaaaaaaaaaaaaaaaaaaaaaaaaaaaatgtagacgtggctgtaaaaaaaaaaaaaaaaaaaaaaaaaaaaaaaaaaaaaaaaaaaaaaaaaaaaaaaaaa

SEQ ID NO: 22 - DNA, 20 bp, synthetic construct
  source 1..20: mol_type = other DNA
aactgtagacgtggctgttt

SEQ ID NO: 23 - DNA, 20 bp, synthetic construct
  source 1..20: mol_type = other DNA
aaaaaaagacgtggaaaatt

SEQ ID NO: 24 - DNA, 20 bp, synthetic construct
  source 1..20: mol_type = other DNA
aaaaaatataaaaaaaaatt

SEQ ID NO: 25 - DNA, 20 bp, synthetic construct
  source 1..20: mol_type = other DNA
acctttcagtggctccattc

SEQ ID NO: 26 - DNA, 20 bp, synthetic construct
  source 1..20: mol_type = other DNA
tatgagctgccattctggtg